European Patent Application EP 4 212 623 A1, published July 19, 2023. Title: A highly active coagulation factor XI mutant, Ala570thr. Applicant: RUIJIN HOSPITAL SHANGHAI JIAOTONG UNIVERSITY SCHOOL OF MEDICINE; WANG Xuefeng; WU Wenman; DING Qiulan. The sequence listing filed with the application follows.

SEQUENCE LISTING (5 sequences)

SEQ ID NO: 1 - DNA, 1878 bp, Artificial Sequence
  Synthesized
tgattttcttatatcaagtggtacatttcattttatttacttcagtttctggtgaatgtgtgactcagttgttgaaggacacctgctttgaaggaggggacattactacggtcttcacaccaagcgccaagtactgccaggtagtctgcacttaccacccaagatgtttactcttcactttcacggcggaatcaccatctgaggatcccacccgatggtttacttgtgtcctgaaagacagtgttacagaaacactgccaagagtgaataggacagcagcgatttctgggtattctttcaagcaatgctcacaccaaataagcgcttgcaacaaagacatttatgtggacctagacatgaagggcataaactataacagctcagttgccaagagtgctcaagaatgccaagaaagatgcacggatgacgtccactgccactttttcacgtacgccacaaggcagtttcccagcctggagcatcgtaacatttgtctactgaagcacacccaaacagggacaccaaccagaataacgaagctcgataaagtggtgtctggattttcactgaaatcctgtgcactttctaatctggcttgtattagggacattttccctaatacggtgtttgcagacagcaacatcgacagtgtcatggctcccgatgcttttgtctgtggccgaatctgcactcatcatcccggttgcttgttttttaccttcttttcccaggaatggcccaaagaatctcaaagaaatctttgtctccttaaaacatctgagagtggattgcccagtacacgcattaaaaagagcaaagctctttctggtttcagtctacaaagctgcaggcacagcatcccagtgttctgccattcttcattttaccatgacactgatttcttgggagaagaactggatattgttgctgcaaaaagtcacgaggcctgccagaaactgtgcaccaatgccgtccgctgccagttttttacctataccccagcccaagcatcctgcaacgaagggaagggcaagtgttacttaaagctttcttcaaacggatctccaactaaaatacttcacgggagaggaggcatctctggatacacattaaggttgtgtaaaatggataatgagtgtaccaccaaaatcaagcccaggatcgttggaggaactgcgtctgttcgtggtgagtggccgtggcaggtgaccctgcacacaacctcacccactcagagacacctgtgtggaggctccatcattggaaaccagtggatattaacagccgctcactgtttctatggggtagagtcacctaagattttgcgtgtctacagtggcattttaaatcaatctgaaataaaagaggacacatctttctttggggttcaagaaataataatccatgatcagtataaaatggcagaaagcgggtatgatattgccttgttgaaactggaaaccacagtgaattacacagattctcaacgacccatatgcctgccttccaaaggagatagaaatgtaatatacactgattgctgggtgactggatgggggtacagaaaactaagagacaaaatacaaaatactctccagaaagccaagatacccttagtgaccaacgaagagtgccagaagagatacagaggacataaaataacccataagatgatctgtgccggctacagggaaggagggaaggacacttgcaagggagattcgggaggccctctgtcctgcaaacacaatgaggtctggcatctggtaggcatcacgagctggggcgaaggctgtgctcaaagggagcggccaggtgtttacaccaacgtggtcgagtacgtggactggattctggagaaaaactcaagcagtgtga

SEQ ID NO: 2 - DNA, 1878 bp, Artificial Sequence
  Synthesized
tgattttcttatatcaagtggtacatttcattttatttacttcagtttctggtgaatgtgtgactcagttgttgaaggacacctgctttgaaggaggggacattactacggtcttcacaccaagcgccaagtactgccaggtagtctgcacttaccacccaagatgtttactcttcactttcacggcggaatcaccatctgaggatcccacccgatggtttacttgtgtcctgaaagacagtgttacagaaacactgccaagagtgaataggacagcagcgatttctgggtattctttcaagcaatgctcacaccaaataagcgcttgcaacaaagacatttatgtggacctagacatgaagggcataaactataacagctcagttgccaagagtgctcaagaatgccaagaaagatgcacggatgacgtccactgccactttttcacgtacgccacaaggcagtttcccagcctggagcatcgtaacatttgtctactgaagcacacccaaacagggacaccaaccagaataacgaagctcgataaagtggtgtctggattttcactgaaatcctgtgcactttctaatctggcttgtattagggacattttccctaatacggtgtttgcagacagcaacatcgacagtgtcatggctcccgatgcttttgtctgtggccgaatctgcactcatcatcccggttgcttgttttttaccttcttttcccaggaatggcccaaagaatctcaaagaaatctttgtctccttaaaacatctgagagtggattgcccagtacacgcattaaaaagagcaaagctctttctggtttcagtctacaaagctgcaggcacagcatcccagtgttctgccattcttcattttaccatgacactgatttcttgggagaagaactggatattgttgctgcaaaaagtcacgaggcctgccagaaactgtgcaccaatgccgtccgctgccagttttttacctataccccagcccaagcatcctgcaacgaagggaagggcaagtgttacttaaagctttcttcaaacggatctccaactaaaatacttcacgggagaggaggcatctctggatacacattaaggttgtgtaaaatggataatgagtgtaccaccaaaatcaagcccaggatcgttggaggaactgcgtctgttcgtggtgagtggccgtggcaggtgaccctgcacacaacctcacccactcagagacacctgtgtggaggctccatcattggaaaccagtggatattaacagccgctcactgtttctatggggtagagtcacctaagattttgcgtgtctacagtggcattttaaatcaatctgaaataaaagaggacacatctttctttggggttcaagaaataataatccatgatcagtataaaatggcagaaagcgggtatgatattgccttgttgaaactggaaaccacagtgaattacacagattctcaacgacccatatgcctgccttccaaaggagatagaaatgtaatatacactgattgctgggtgactggatgggggtacagaaaactaagagacaaaatacaaaatactctccagaaagccaagatacccttagtgaccaacgaagagtgccagaagagatacagaggacataaaataacccataagatgatctgtgccggctacagggaaggagggaaggacacctgcaagggagattcgggaggccctctgtcctgcaaacacaatgaggtctggcatctggtaggcatcacgagctggggcgaaggctgtgctcaaagggagcggccaggtgtttacaccaacgtggtcgagtacgtggactggattctggagaaaaactcaagcagtgtga

SEQ ID NO: 3 - DNA, 1878 bp, Artificial Sequence
  Synthesized
tgattttcttatatcaagtggtacatttcattttatttacttcagtttctggtgaatgtgtgactcagttgttgaaggacacctgctttgaaggaggggacattactacggtcttcacaccaagcgccaagtactgccaggtagtctgcacttaccacccaagatgtttactcttcactttcacggcggaatcaccatctgaggatcccacccgatggtttacttgtgtcctgaaagacagtgttacagaaacactgccaagagtgaataggacagcagcgatttctgggtattctttcaagcaatgctcacaccaaataagcgcttgcaacaaagacatttatgtggacctagacatgaagggcataaactataacagctcagttgccaagagtgctcaagaatgccaagaaagatgcacggatgacgtccactgccactttttcacgtacgccacaaggcagtttcccagcctggagcatcgtaacatttgtctactgaagcacacccaaacagggacaccaaccagaataacgaagctcgataaagtggtgtctggattttcactgaaatcctgtgcactttctaatctggcttgtattagggacattttccctaatacggtgtttgcagacagcaacatcgacagtgtcatggctcccgatgcttttgtctgtggccgaatctgcactcatcatcccggttgcttgttttttaccttcttttcccaggaatggcccaaagaatctcaaagaaatctttgtctccttaaaacatctgagagtggattgcccagtacacgcattaaaaagagcaaagctctttctggtttcagtctacaaagctgcaggcacagcatcccagtgttctgccattcttcattttaccatgacactgatttcttgggagaagaactggatattgttgctgcaaaaagtcacgaggcctgccagaaactgtgcaccaatgccgtccgctgccagttttttacctataccccagcccaagcatcctgcaacgaagggaagggcaagtgttacttaaagctttcttcaaacggatctccaactaaaatacttcacgggagaggaggcatctctggatacacattaaggttgtgtaaaatggataatgagtgtaccaccaaaatcaagcccaggatcgttggaggaactgcgtctgttcgtggtgagtggccgtggcaggtgaccctgcacacaacctcacccactcagagacacctgtgtggaggctccatcattggaaaccagtggatattaacagccgctcactgtttctatggggtagagtcacctaagattttgcgtgtctacagtggcattttaaatcaatctgaaataaaagaggacacatctttctttggggttcaagaaataataatccatgatcagtataaaatggcagaaagcgggtatgatattgccttgttgaaactggaaaccacagtgaattacacagattctcaacgacccatatgcctgccttccaaaggagatagaaatgtaatatacactgattgctgggtgactggatgggggtacagaaaactaagagacaaaatacaaaatactctccagaaagccaagatacccttagtgaccaacgaagagtgccagaagagatacagaggacataaaataacccataagatgatctgtgccggctacagggaaggagggaaggacacgtgcaagggagattcgggaggccctctgtcctgcaaacacaatgaggtctggcatctggtaggcatcacgagctggggcgaaggctgtgctcaaagggagcggccaggtgtttacaccaacgtggtcgagtacgtggactggattctggagaaaaactcaagcagtgtga

SEQ ID NO: 4 - DNA, 1878 bp, Artificial Sequence
  Synthesized
tgattttcttatatcaagtggtacatttcattttatttacttcagtttctggtgaatgtgtgactcagttgttgaaggacacctgctttgaaggaggggacattactacggtcttcacaccaagcgccaagtactgccaggtagtctgcacttaccacccaagatgtttactcttcactttcacggcggaatcaccatctgaggatcccacccgatggtttacttgtgtcctgaaagacagtgttacagaaacactgccaagagtgaataggacagcagcgatttctgggtattctttcaagcaatgctcacaccaaataagcgcttgcaacaaagacatttatgtggacctagacatgaagggcataaactataacagctcagttgccaagagtgctcaagaatgccaagaaagatgcacggatgacgtccactgccactttttcacgtacgccacaaggcagtttcccagcctggagcatcgtaacatttgtctactgaagcacacccaaacagggacaccaaccagaataacgaagctcgataaagtggtgtctggattttcactgaaatcctgtgcactttctaatctggcttgtattagggacattttccctaatacggtgtttgcagacagcaacatcgacagtgtcatggctcccgatgcttttgtctgtggccgaatctgcactcatcatcccggttgcttgttttttaccttcttttcccaggaatggcccaaagaatctcaaagaaatctttgtctccttaaaacatctgagagtggattgcccagtacacgcattaaaaagagcaaagctctttctggtttcagtctacaaagctgcaggcacagcatcccagtgttctgccattcttcattttaccatgacactgatttcttgggagaagaactggatattgttgctgcaaaaagtcacgaggcctgccagaaactgtgcaccaatgccgtccgctgccagttttttacctataccccagcccaagcatcctgcaacgaagggaagggcaagtgttacttaaagctttcttcaaacggatctccaactaaaatacttcacgggagaggaggcatctctggatacacattaaggttgtgtaaaatggataatgagtgtaccaccaaaatcaagcccaggatcgttggaggaactgcgtctgttcgtggtgagtggccgtggcaggtgaccctgcacacaacctcacccactcagagacacctgtgtggaggctccatcattggaaaccagtggatattaacagccgctcactgtttctatggggtagagtcacctaagattttgcgtgtctacagtggcattttaaatcaatctgaaataaaagaggacacatctttctttggggttcaagaaataataatccatgatcagtataaaatggcagaaagcgggtatgatattgccttgttgaaactggaaaccacagtgaattacacagattctcaacgacccatatgcctgccttccaaaggagatagaaatgtaatatacactgattgctgggtgactggatgggggtacagaaaactaagagacaaaatacaaaatactctccagaaagccaagatacccttagtgaccaacgaagagtgccagaagagatacagaggacataaaataacccataagatgatctgtgccggctacagggaaggagggaaggacacatgcaagggagattcgggaggccctctgtcctgcaaacacaatgaggtctggcatctggtaggcatcacgagctggggcgaaggctgtgctcaaagggagcggccaggtgtttacaccaacgtggtcgagtacgtggactggattctggagaaaaactcaagcagtgtga

SEQ ID NO: 5 - protein, 625 aa, Artificial Sequence
  Synthesized
MIFLYQVVHFILFTSVSGECVTQLLKDTCFEGGDITTVFTPSAKYCQVVCTYHPRCLLFTFTAESPSEDPTRWFTCVLKDSVTETLPRVNRTAAISGYSFKQCSHQISACNKDIYVDLDMKGINYNSSVAKSAQECQERCTDDVHCHFFTYATRQFPSLEHRNICLLKHTQTGTPTRITKLDKVVSGFSLKSCALSNLACIRDIFPNTVFADSNIDSVMAPDAFVCGRICTHHPGCLFFTFFSQEWPKESQRNLCLLKTSESGLPSTRIKKSKALSGFSLQSCRHSIPVFCHSSFYHDTDFLGEELDIVAAKSHEACQKLCTNAVRCQFFTYTPAQASCNEGKGKCYLKLSSNGSPTKILHGRGGISGYTLRLCKMDNECTTKIKPRIVGGTASVRGEWPWQVTLHTTSPTQRHLCGGSIIGNQWILTAAHCFYGVESPKILRVYSGILNQSEIKEDTSFFGVQEIIIHDQYKMAESGYDIALLKLETTVNYTDSQRPICLPSKGDRNVIYTDCWVTGWGYRKLRDKIQNTLQKAKIPLVTNEECQKRYRGHKITHKMICAGYREGGKDTCKGDSGGPLSCKHNEVWHLVGITSWGEGCAQRERPGVYTNVVEYVDWILEKTQAV